European Patent Specification EP 3 590 958 B1, published May 6, 2026. Title: TCR LIBRARIES. Applicant: Immunocore Limited Adaptimmune Limited. The sequence listing filed with the application follows.

SEQUENCE LISTING (9 sequences)

SEQ ID NO: 1 - DNA, 20 bp, homo sapiens
cattttcagggatagcaagc

SEQ ID NO: 2 - DNA, 48 bp, homo sapiens
ttctattctcacagcgcgaatgctggtgtcactcagaccccaaaattc

SEQ ID NO: 3 - DNA, 41 bp, homo sapiens
gcccagccggccatggcccagaaggaggtggagcagaattc

SEQ ID NO: 4 - DNA, 41 bp, homo sapiens
gcccagccggccatggccaaacaggaggtgacgcagattcc

SEQ ID NO: 5 - DNA, 22 bp, homo sapiens
gagtctctcagctggtacacgg

SEQ ID NO: 6 - DNA, 20 bp, homo sapiens
agtgtggccttttgggtgtg

SEQ ID NO: 7 - DNA, 22 bp, homo sapiens
ccgtgtaccagctgagagactc

SEQ ID NO: 8 - DNA, 21 bp, homo sapiens
gcgcgctgtgagaatagaaag

SEQ ID NO: 9 - DNA, 20 bp, homo sapiens
cacacccaaaaggccacact